European Patent Specification EP 3 548 510 B1, published October 2, 2024. Title: COMPOUNDS USEFUL FOR THE TREATMENT AND/OR CARE OF THE SKIN, HAIR, NAILS AND/OR MUCOUS MEMBRANES. Applicant: Lubrizol Advanced Materials, Inc. Application EP16382581.3. The sequence listing filed with the application follows.

SEQUENCE LISTING (50 sequences)

SEQ ID NO: 1 - protein, 12 aa, Artifical Sequence
  SITE (1)..(1): Xaa is any amino acid or no amino acid
  SITE (2)..(2): Xaa is any amino acid or no amino acid
  SITE (3)..(3): Xaa is Glu, Asp, Gln or Asn
  SITE (4)..(4): Xaa is Glu, Asp or Gln
  SITE (5)..(5): Xaa is Met, Leu or Ile
  SITE (6)..(6): Xaa is Gln, Glu, Asn or Asp
  SITE (7)..(7): Xaa is Arg or Lys
  SITE (8)..(8): Xaa is Arg, Lys or His
  SITE (9)..(9): Xaa is no amino acid or Ala, Ser, Gly, Thr, Pro, Glu, Lys or Val
  SITE (10)..(10): Xaa is no amino acid or Asp, Glu, Asn or Gln
  SITE (11)..(11): Xaa is any amino acid or no amino acid
  SITE (12)..(12): Xaa is any amino acid or no amino acid
XXXXXXXXXXXX

SEQ ID NO: 2 - protein, 6 aa, Artificial Sequence
  synthetic peptide
EEMQRR

SEQ ID NO: 3 - protein, 7 aa, Artificial Sequence
  synthetic peptide
EEMQRRA

SEQ ID NO: 4 - protein, 8 aa, Artificial sequence
  synthetic peptide
EEMQRRAD

SEQ ID NO: 5 - protein, 8 aa, Artificial sequence
  synthetic peptide
DEMQRRAD

SEQ ID NO: 6 - protein, 8 aa, Artificial sequence
  synthetic peptide
QEMQRRAD

SEQ ID NO: 7 - protein, 8 aa, Artificial sequence
  synthetic peptide
EELQRRAD

SEQ ID NO: 8 - protein, 8 aa, Artificial sequence
  synthetic peptide
EEMERRAD

SEQ ID NO: 9 - protein, 8 aa, Artificial sequence
  synthetic peptide
EEMNRRAD

SEQ ID NO: 10 - protein, 8 aa, Artificial sequence
  synthetic peptide
EEMDRRAD

SEQ ID NO: 11 - protein, 8 aa, synthetic peptide
EEMQRKAD

SEQ ID NO: 12 - protein, 8 aa, Artificial sequence
  synthetic peptide
EEMQRRSD

SEQ ID NO: 13 - protein, 8 aa, Artificial sequence
  synthetic peptide
EEMQRRGD

SEQ ID NO: 14 - protein, 8 aa, Artificial sequence
  synthetic peptide
EEMQRRAE

SEQ ID NO: 15 - protein, 8 aa, Artificial Sequence
  synthetic peptide
EEMQRRAN

SEQ ID NO: 16 - protein, 8 aa, Artificial sequence
  synthetic peptide
EEMQRRAQ

SEQ ID NO: 17 - protein, 8 aa, Artificial sequence
  synthetic peptide
EEMQRHAD

SEQ ID NO: 18 - protein, 8 aa, Artificial sequence
  synthetic peptide
EEMQRRTD

SEQ ID NO: 19 - protein, 8 aa, Artificial sequence
  synthetic peptide
EEMQRRPD

SEQ ID NO: 20 - protein, 8 aa, Artificial sequence
  synthetic peptide
EEMQRRED

SEQ ID NO: 21 - protein, 8 aa, Artificial sequence
  synthetic peptide
EEMQRRKD

SEQ ID NO: 22 - protein, 7 aa, Artificial sequence
  synthetic peptide
EEMQRRS

SEQ ID NO: 23 - protein, 7 aa, Artificial sequence
  synthetic peptide
EEMQRRG

SEQ ID NO: 24 - protein, 7 aa, Artificial sequence
  synthetic peptide
EEMERRA

SEQ ID NO: 25 - protein, 7 aa, Artificial sequence
  synthetic peptide
DEMERRA

SEQ ID NO: 26 - protein, 7 aa, Artificial sequence
  synthetic peptide
EEMQRRT

SEQ ID NO: 27 - protein, 7 aa, Artificial sequence
  synthetic peptide
EEMDRRA

SEQ ID NO: 28 - protein, 7 aa, Artificial sequence
  synthetic peptide
NEMQRRA

SEQ ID NO: 29 - protein, 7 aa, Artificial sequence
  synthetic peptide
EEMQRRV

SEQ ID NO: 30 - protein, 6 aa, Artificial sequence
  synthetic peptide
EEMQRK

SEQ ID NO: 31 - protein, 6 aa, Artificial sequence
  synthetic peptide
EEMQKR

SEQ ID NO: 32 - protein, 6 aa, Artificial sequence
  synthetic peptide
EEMERR

SEQ ID NO: 33 - protein, 6 aa, Artificial sequence
  synthetic peptide
EEMNRR

SEQ ID NO: 34 - protein, 6 aa, Artificial sequence
  synthetic peptide
EDMQRR

SEQ ID NO: 35 - protein, 6 aa, Artificial sequence
  synthetic peptide
EQMQRR

SEQ ID NO: 36 - protein, 6 aa, Artificial sequence
  synthetic peptide
DEMQRR

SEQ ID NO: 37 - protein, 6 aa, Artificial sequence
  synthetic peptide
QEMQRR

SEQ ID NO: 38 - protein, 6 aa, Artificial sequence
  synthetic peptide
EEMQRH

SEQ ID NO: 39 - protein, 6 aa, Artificial sequence
  synthetic peptide
EEMQKK

SEQ ID NO: 40 - protein, 6 aa, Artificial sequence
  synthetic peptide
EEIERR

SEQ ID NO: 41 - protein, 6 aa, Artificial sequence
  synthetic peptide
EELQRR

SEQ ID NO: 42 - protein, 10 aa, Artificial sequence
  synthetic peptide
ELEEMQRRAD

SEQ ID NO: 43 - protein, 9 aa, Artificial sequence
  synthetic peptide
ELEEMQRRA

SEQ ID NO: 44 - protein, 8 aa, Artificial sequence
  synthetic peptide
ELEEMQRR

SEQ ID NO: 45 - protein, 10 aa, Artificial sequence
  synthetic peptide
LEEMQRRADQ

SEQ ID NO: 46 - protein, 9 aa, Artificial sequence
  synthetic peptide
LEEMQRRAD

SEQ ID NO: 47 - protein, 8 aa, Artificial sequence
  synthetic peptide
LEEMQRRA

SEQ ID NO: 48 - protein, 7 aa, Artificial sequence
  synthetic peptide
LEEMQRR

SEQ ID NO: 49 - protein, 10 aa, Artificial sequence
  synthetic peptide
EEMQRRADQL

SEQ ID NO: 50 - protein, 9 aa, Artificial sequence
  synthetic peptide
EEMQRRADQ